European Patent Application EP 4 785 957 A1, published August 5, 2026. Title: 一种抗破伤风毒素抗体在预防或治疗破伤风中的应用. Applicant: 珠海泰诺麦博制药股份有限公司. The sequence listing filed with the application follows.

SEQUENCE LISTING (10 sequences)

SEQ ID NO: 1 - protein, 8 aa, synthetic construct
GGPFTGSY

SEQ ID NO: 2 - protein, 7 aa, synthetic construct
VSQSGST

SEQ ID NO: 3 - protein, 12 aa, synthetic construct
ARLTKHYINSAY

SEQ ID NO: 4 - protein, 118 aa, synthetic construct
QVQLQESGAGLVKPSETLSLTCGVAGGPFTGSYLSWIRQPPGKGLEWIGEVSQSGSTSYNPSLKSRVTISVDTSKSQFSLKLSSVTAADTAVYYCARLTKHYINSAYWGQGTLVTVSS

SEQ ID NO: 5 - protein, 448 aa, synthetic construct
QVQLQESGAGLVKPSETLSLTCGVAGGPFTGSYLSWIRQPPGKGLEWIGEVSQSGSTSYNPSLKSRVTISVDTSKSQFSLKLSSVTAADTAVYYCARLTKHYINSAYWGQGTLVTVSSASTKGPSVFPLAPSSKSTSGGTAALGCLVKDYFPEPVTVSWNSGALTSGVHTFPAVLQSSGLYSLSSVVTVPSSSLGTQTYICNVNHKPSNTKVDKRVEPKSCDKTHTCPPCPAPELLGGPSVFLFPPKPKDTLMISRTPEVTCVVVDVSHEDPEVKFNWYVDGVEVHNAKTKPREEQYNSTYRVVSVLTVLHQDWLNGKEYKCKVSNKALPAPIEKTISKAKGQPREPQVYTLPPSREEMTKNQVSLTCLVKGFYPSDIAVEWESNGQPENNYKTTPPVLDSDGSFFLYSKLTVDKSRWQQGNVFSCSVMHEALHNHYTQKSLSLSPGK

SEQ ID NO: 6 - protein, 6 aa, synthetic construct
QIIGSW

SEQ ID NO: 7 - skipped

SEQ ID NO: 8 - protein, 9 aa, synthetic construct
QQYNSYPYT

SEQ ID NO: 9 - protein, 107 aa, synthetic construct
DIQMTQSPSILSASVGDRVTITCRASQIIGSWLAWYQQKPGKAPTLVIYKASRLDSGVPSRFSGTESGTEFTLTISSLQPDDFATYYCQQYNSYPYTFGQGTKLEIK

SEQ ID NO: 10 - protein, 214 aa, synthetic construct
DIQMTQSPSILSASVGDRVTITCRASQIIGSWLAWYQQKPGKAPTLVIYKASRLDSGVPSRFSGTESGTEFTLTISSLQPDDFATYYCQQYNSYPYTFGQGTKLEIKRTVAAPSVFIFPPSDEQLKSGTASVVCLLNNFYPREAKVQWKVDNALQSGNSQESVTEQDSKDSTYSLSSTLTLSKADYEKHKVYACEVTHQGLSSPVTKSFNRGEC